European Patent Application EP 4 471 057 A1, published December 4, 2024. Title: Anti-hCXCL1 antibody. Applicant: 株式会社カイオム・バイオサイエンス. The sequence listing filed with the application follows.

SEQUENCE LISTING (82 sequences)

SEQ ID NO: 1 - protein, 116 aa, Mus musculus
QVQLKESGPVLVAPSQSLSITCSVSGFSSTTYGVHWVRQPPGQGLEWLGVIWAGGSTNYNSALMSRLSISKDNSKSQVFLKMNSLQTDDTAMYYCATQYHYPFAYWGQGTLVTVSA

SEQ ID NO: 2 - protein, 5 aa, Mus musculus
TYGVH

SEQ ID NO: 3 - protein, 16 aa, Mus musculus
VIWAGGSTNYNSALMS

SEQ ID NO: 4 - protein, 8 aa, Mus musculus
QYHYPFAY

SEQ ID NO: 5 - protein, 107 aa, Mus musculus
NIVMTQSPKSMSMSVGERVTLSCKASENVGIYVSWYQQKPEQSPKLMIYGASNRNTGVPDRFTGSGSATDFTLTISSVQAEDLADYYCGQSYSYPLTFGAGTKLELK

SEQ ID NO: 6 - protein, 11 aa, Mus musculus
KASENVGIYVS

SEQ ID NO: 7 - protein, 7 aa, Mus musculus
GASNRNT

SEQ ID NO: 8 - protein, 9 aa, Mus musculus
GQSYSYPLT

SEQ ID NO: 9 - protein, 123 aa, Mus musculus
QVTLKESGPGILKPSQTLSLTCSFSGFSLSTSGMGVDWIRQPSGKGLEWLAHIWWDDDKYYNPSLKSQLTISKDTSRNQVFLKITSVDTADTATYYCARSYGYDMDYYAMDYWGQGTSVTVSS

SEQ ID NO: 10 - protein, 7 aa, Mus musculus
TSGMGVD

SEQ ID NO: 11 - protein, 16 aa, Mus musculus
HIWWDDDKYYNPSLKS

SEQ ID NO: 12 - protein, 13 aa, Mus musculus
SYGYDMDYYAMDY

SEQ ID NO: 13 - protein, 108 aa, Mus musculus
DIQMTQSPSSLSASLGERVSLTCRASQEISGYLSWLQQKPDGTIKRLIYAASTLDSGVPKRFSGSRSGSDYSLTISSLESEDFADYYCLQYASYPPWTFGGGTKLEIK

SEQ ID NO: 14 - protein, 11 aa, Mus musculus
RASQEISGYLS

SEQ ID NO: 15 - protein, 7 aa, Mus musculus
AASTLDS

SEQ ID NO: 16 - protein, 10 aa, Mus musculus
LQYASYPPWT

SEQ ID NO: 17 - protein, 119 aa, Mus musculus
QVQLQQSGAELVRPGSSVKISCKASGYAFSDYWMNWVKQRPGQGLEWIGQIYPGDGDTNYNGKFKGKGTLTADKSSSTAYMQLNSLTSEDSAVYFCARERDYDVAMDYWGQGTSVTVSS

SEQ ID NO: 18 - protein, 5 aa, Mus musculus
DYWMN

SEQ ID NO: 19 - protein, 17 aa, Mus musculus
QIYPGDGDTNYNGKFKG

SEQ ID NO: 20 - protein, 10 aa, Mus musculus
ERDYDVAMDY

SEQ ID NO: 21 - protein, 107 aa, Mus musculus
DIQMTQSPSSLSASLGGKVTITCKASQDINKYIAWFQHKPGKGPRLVIHYTSILQPGIPSRFSGVGSGRDYSFSIRNLEPEDIATYYCLQYDNLPWTFGGGTKLEIK

SEQ ID NO: 22 - protein, 11 aa, Mus musculus
KASQDINKYIA

SEQ ID NO: 23 - protein, 7 aa, Mus musculus
YTSILQP

SEQ ID NO: 24 - protein, 9 aa, Mus musculus
LQYDNLPWT

SEQ ID NO: 25 - protein, 125 aa, Gallus gallus
EVQLLESGGGLVQPGGSLRLSCAASGFTFSELSMSWVRQAPGKGLEWVSAISGSGGSTYYADSVKGRFTISRDNSKNTLYLQMNSLRAEDTAVYYCAREGGRLEPYYYYYAMDVWGQGTPVTVSS

SEQ ID NO: 26 - protein, 5 aa, Gallus gallus
ELSMS

SEQ ID NO: 27 - protein, 17 aa, Gallus gallus
AISGSGGSTYYADSVKG

SEQ ID NO: 28 - protein, 16 aa, Gallus gallus
EGGRLEPYYYYYAMDV

SEQ ID NO: 29 - protein, 107 aa, Gallus gallus
DIQMTQSPSSLSASVGDRVTITCRASQSISDNLHWYQQKPGKAPKLLIYDASNLESGVPSRFSGSGSGTDFTLTINSLQPEDFATYYCQQYYSTPLTFGQGTKLEIK

SEQ ID NO: 30 - protein, 11 aa, Gallus gallus
RASQSISDNLH

SEQ ID NO: 31 - protein, 7 aa, Gallus gallus
DASNLES

SEQ ID NO: 32 - protein, 9 aa, Gallus gallus
QQYYSTPLT

SEQ ID NO: 33 - protein, 116 aa, synthetic construct
  REGION 1..116: note = Recombinant peptide
QVQLKESGPVLVAPSQSLSITCSVSGFSSTTYGVHWVRQPPGQGLEWLGVIWAGGSTNYNAALMSRLSISKDNSKSQVFLKMNSLQTDDTAMYYCATQYHYPFAYWGQGTLVTVSA

SEQ ID NO: 34 - protein, 16 aa, synthetic construct
  REGION 1..16: note = Recombinant peptide
VIWAGGSTNYNAALMS

SEQ ID NO: 35 - protein, 108 aa, synthetic construct
  REGION 1..108: note = Recombinant peptide
DIQMTQSPSSLSASLGERVSLTCRASQEISGYLSWLQQKPDGTIKRLIYAASTLSSGVPKRFSGSRSGSDYSLTISSLESEDFADYYCLQYASYPPWTFGGGTKLEIK

SEQ ID NO: 36 - protein, 7 aa, synthetic construct
  REGION 1..7: note = Recombinant peptide
AASTLSS

SEQ ID NO: 37 - protein, 108 aa, synthetic construct
  REGION 1..108: note = Recombinant peptide
DIQMTQSPSSLSASLGERVSLTCRASQEISGYLSWLQQKPDGTIKRLIYAASTLESGVPKRFSGSRSGSDYSLTISSLESEDFADYYCLQYASYPPWTFGGGTKLEIK

SEQ ID NO: 38 - protein, 7 aa, synthetic construct
  REGION 1..7: note = Recombinant peptide
AASTLES

SEQ ID NO: 39 - protein, 108 aa, synthetic construct
  REGION 1..108: note = Recombinant peptide
DIQMTQSPSSLSASLGERVSLTCRASQEISGYLSWLQQKPDGTIKRLIYAASTLDAGVPKRFSGSRSGSDYSLTISSLESEDFADYYCLQYASYPPWTFGGGTKLEIK

SEQ ID NO: 40 - protein, 7 aa, synthetic construct
  REGION 1..7: note = Recombinant peptide
AASTLDA

SEQ ID NO: 41 - protein, 119 aa, synthetic construct
  REGION 1..119: note = Recombinant peptide
QVQLQQSGAELVRPGSSVKISCKASGYAFSDYWMNWVKQRPGQGLEWIGQIYPGSGDTNYNGKFKGKGTLTADKSSSTAYMQLNSLTSEDSAVYFCARERDYDVAMDYWGQGTSVTVSS

SEQ ID NO: 42 - protein, 17 aa, synthetic construct
  REGION 1..17: note = Recombinant peptide
QIYPGSGDTNYNGKFKG

SEQ ID NO: 43 - protein, 119 aa, synthetic construct
  REGION 1..119: note = Recombinant peptide
QVQLQQSGAELVRPGSSVKISCKASGYAFSDYWMNWVKQRPGQGLEWIGQIYPGEGDTNYNGKFKGKGTLTADKSSSTAYMQLNSLTSEDSAVYFCARERDYDVAMDYWGQGTSVTVSS

SEQ ID NO: 44 - protein, 17 aa, synthetic construct
  REGION 1..17: note = Recombinant peptide
QIYPGEGDTNYNGKFKG

SEQ ID NO: 45 - protein, 119 aa, synthetic construct
  REGION 1..119: note = Recombinant peptide
QVQLQQSGAELVRPGSSVKISCKASGYAFSDYWMNWVKQRPGQGLEWIGQIYPGDADTNYNGKFKGKGTLTADKSSSTAYMQLNSLTSEDSAVYFCARERDYDVAMDYWGQGTSVTVSS

SEQ ID NO: 46 - protein, 17 aa, synthetic construct
  REGION 1..17: note = Recombinant peptide
QIYPGDADTNYNGKFKG

SEQ ID NO: 47 - protein, 119 aa, synthetic construct
  REGION 1..119: note = Recombinant peptide
QVQLQQSGAELVRPGSSVKISCKASGYAFSDYWMNWVKQRPGQGLEWIGQIYPGDGDTNYSGKFKGKGTLTADKSSSTAYMQLNSLTSEDSAVYFCARERDYDVAMDYWGQGTSVTVSS

SEQ ID NO: 48 - protein, 17 aa, synthetic construct
  REGION 1..17: note = Recombinant peptide
QIYPGDGDTNYSGKFKG

SEQ ID NO: 49 - protein, 119 aa, synthetic construct
  REGION 1..119: note = Recombinant peptide
QVQLQQSGAELVRPGSSVKISCKASGYAFSDYWMNWVKQRPGQGLEWIGQIYPGDGDTNYNAKFKGKGTLTADKSSSTAYMQLNSLTSEDSAVYFCARERDYDVAMDYWGQGTSVTVSS

SEQ ID NO: 50 - protein, 17 aa, synthetic construct
  REGION 1..17: note = Recombinant peptide
QIYPGDGDTNYNAKFKG

SEQ ID NO: 51 - protein, 119 aa, synthetic construct
  REGION 1..119: note = Recombinant peptide
QVQLQQSGAELVRPGSSVKISCKASGYAFSDYWMNWVKQRPGQGLEWIGQIYPGSGDTNYSGKFKGKGTLTADKSSSTAYMQLNSLTSEDSAVYFCARERDYDVAMDYWGQGTSVTVSS

SEQ ID NO: 52 - protein, 17 aa, synthetic construct
  REGION 1..17: note = Recombinant peptide
QIYPGSGDTNYSGKFKG

SEQ ID NO: 53 - protein, 119 aa, synthetic construct
  REGION 1..119: note = Recombinant peptide
QVQLQQSGAELVRPGSSVKISCKASGYAFSDYWMNWVKQRPGQGLEWIGQIYPGSGDTNYNAKFKGKGTLTADKSSSTAYMQLNSLTSEDSAVYFCARERDYDVAMDYWGQGTSVTVSS

SEQ ID NO: 54 - protein, 17 aa, synthetic construct
  REGION 1..17: note = Recombinant peptide
QIYPGSGDTNYNAKFKG

SEQ ID NO: 55 - protein, 119 aa, synthetic construct
  REGION 1..119: note = Recombinant peptide
QVQLQQSGAELVRPGSSVKISCKASGYAFSDYWMNWVKQRPGQGLEWIGQIYPGEGDTNYSGKFKGKGTLTADKSSSTAYMQLNSLTSEDSAVYFCARERDYDVAMDYWGQGTSVTVSS

SEQ ID NO: 56 - protein, 17 aa, synthetic construct
  REGION 1..17: note = Recombinant peptide
QIYPGEGDTNYSGKFKG

SEQ ID NO: 57 - protein, 119 aa, synthetic construct
  REGION 1..119: note = Recombinant peptide
QVQLQQSGAELVRPGSSVKISCKASGYAFSDYWMNWVKQRPGQGLEWIGQIYPGEGDTNYNAKFKGKGTLTADKSSSTAYMQLNSLTSEDSAVYFCARERDYDVAMDYWGQGTSVTVSS

SEQ ID NO: 58 - protein, 17 aa, synthetic construct
  REGION 1..17: note = Recombinant peptide
QIYPGEGDTNYNAKFKG

SEQ ID NO: 59 - protein, 119 aa, synthetic construct
  REGION 1..119: note = Recombinant peptide
QVQLQQSGAELVRPGSSVKISCKASGYAFSDYWMNWVKQRPGQGLEWIGQIYPGDADTNYSGKFKGKGTLTADKSSSTAYMQLNSLTSEDSAVYFCARERDYDVAMDYWGQGTSVTVSS

SEQ ID NO: 60 - protein, 17 aa, synthetic construct
  REGION 1..17: note = Recombinant peptide
QIYPGDADTNYSGKFKG

SEQ ID NO: 61 - protein, 119 aa, synthetic construct
  REGION 1..119: note = Recombinant peptide
QVQLQQSGAELVRPGSSVKISCKASGYAFSDYWMNWVKQRPGQGLEWIGQIYPGDADTNYNAKFKGKGTLTADKSSSTAYMQLNSLTSEDSAVYFCARERDYDVAMDYWGQGTSVTVSS

SEQ ID NO: 62 - protein, 17 aa, synthetic construct
  REGION 1..17: note = Recombinant peptide
QIYPGDADTNYNAKFKG

SEQ ID NO: 63 - protein, 125 aa, synthetic construct
  REGION 1..125: note = Recombinant peptide
EVQLLESGGGLVQPGGSLRLSCAASGFTFSELSMSWVRQAPGKGLEWVSAISGSGGSTYYASSVKGRFTISRDNSKNTLYLQMNSLRAEDTAVYYCAREGGRLEPYYYYYAMDVWGQGTPVTVSS

SEQ ID NO: 64 - protein, 17 aa, synthetic construct
  REGION 1..17: note = Recombinant peptide
AISGSGGSTYYASSVKG

SEQ ID NO: 65 - protein, 125 aa, synthetic construct
  REGION 1..125: note = Recombinant peptide
EVQLLESGGGLVQPGGSLRLSCAASGFTFSELSMSWVRQAPGKGLEWVSAISGSGGSTYYADAVKGRFTISRDNSKNTLYLQMNSLRAEDTAVYYCAREGGRLEPYYYYYAMDVWGQGTPVTVSS

SEQ ID NO: 66 - protein, 17 aa, synthetic construct
  REGION 1..17: note = Recombinant peptide
AISGSGGSTYYADAVKG

SEQ ID NO: 67 - protein, 107 aa, synthetic construct
  REGION 1..107: note = Recombinant peptide
DIQMTQSPSSLSASVGDRVTITCRASQSISDNLHWYQQKPGKAPKLLIYDASNLESGVPSRFSGSGSGTDFTLTISSLQPEDFATYYCQQYYSTPLTFGQGTKLEIK

SEQ ID NO: 68 - protein, 116 aa, synthetic construct
  REGION 1..116: note = Recombinant peptide
QVTLKESGPVLVKPTETLTLTCTVSGFSSTTYGVHWVRQPPGKALEWLGVIWAGGSTNYNAALMSRLTISKDTSKSQVVLTMTNMDPVDTATYYCATQYHYPFAYWGQGTLVTVSS

SEQ ID NO: 69 - protein, 116 aa, synthetic construct
  REGION 1..116: note = Recombinant peptide
QVTLKESGPVLVKPTETLTLTCTVSGFSSTTYGVHWVRQPPGKALEWLGVIWAGGSTNYNAALMSRLTISKDNSKSQVVLTMTNMDPVDTATYYCATQYHYPFAYWGQGTLVTVSS

SEQ ID NO: 70 - protein, 107 aa, synthetic construct
  REGION 1..107: note = Recombinant peptide
DIQMTQSPSSLSASVGDRVTITCKASENVGIYVSWYQQKPGKAPKLMIYGASNRNTGVPSRFSGSGSGTDFTLTISSLQPEDFATYYCGQSYSYPLTFGGGTKVEIK

SEQ ID NO: 71 - protein, 107 aa, synthetic construct
  REGION 1..107: note = Recombinant peptide
DIQMTQSPSSLSASVGDRVTITCKASENVGIYVSWYQQKPGKAPKLMIYGASNRNTGVPSRFSGSGSATDFTLTISSLQPEDFATYYCGQSYSYPLTFGGGTKVEIK

SEQ ID NO: 72 - protein, 123 aa, synthetic construct
  REGION 1..123: note = Recombinant peptide
QVTLKESGPALVKPTQTLTLTCTFSGFSLSTSGMGVDWIRQPPGKALEWLAHIWWDDDKYYNPSLKSQLTISKDTSKNQVVLTMTNMDPVDTATYYCARSYGYDMDYYAMDYWGQGTTVTVSS

SEQ ID NO: 73 - protein, 123 aa, synthetic construct
  REGION 1..123: note = Recombinant peptide
QVTLKESGPALVKPTQTLTLTCTFSGFSLSTSGMGVDWIRQPPGKGLEWLAHIWWDDDKYYNPSLKSQLTISKDTSKNQVVLTMTNMDPVDTATYYCARSYGYDMDYYAMDYWGQGTTVTVSS

SEQ ID NO: 74 - protein, 108 aa, synthetic construct
  REGION 1..108: note = Recombinant peptide
DIQMTQSPSSLSASVGDRVTITCRASQEISGYLSWLQQKPGKAPKRLIYAASTLSSGVPSRFSGSGSGTDFTLTISSLQPEDFATYYCLQYASYPPWTFGGGTKVEIK

SEQ ID NO: 75 - protein, 108 aa, synthetic construct
  REGION 1..108: note = Recombinant peptide
DIQMTQSPSSLSASVGDRVTITCRASQEISGYLSWLQQKPGKAPKRLIYAASTLSSGVPSRFSGSGSGTDYTLTISSLQPEDFATYYCLQYASYPPWTFGGGTKVEIK

SEQ ID NO: 76 - protein, 119 aa, synthetic construct
  REGION 1..119: note = Recombinant peptide
QVQLVQSGAEVKKPGSSVKVSCKASGYAFSDYWMNWVRQAPGQGLEWIGQIYPGSGDTNYNAKFKGKGTITADKSTSTAYMELSSLRSEDTAVYYCARERDYDVAMDYWGQGTTVTVSS

SEQ ID NO: 77 - protein, 119 aa, synthetic construct
  REGION 1..119: note = Recombinant peptide
QVQLVQSGAEVKKPGSSVKVSCKASGYAFSDYWMNWVRQAPGQGLEWIGQIYPGSGDTNYNAKFKGKGTLTADKSTSTAYMELSSLRSEDTAVYYCARERDYDVAMDYWGQGTTVTVSS

SEQ ID NO: 78 - protein, 107 aa, synthetic construct
  REGION 1..107: note = Recombinant peptide
DIQMTQSPSSLSASVGDRVTITCKASQDINKYIAWFQQKPGKAPKLVIHYTSILQPGVPSRFSGSGSGTDYTFTISSLQPEDIATYYCLQYDNLPWTFGGGTKVEIK

SEQ ID NO: 79 - protein, 107 aa, synthetic construct
  REGION 1..107: note = Recombinant peptide
DIQMTQSPSSLSASVGDRVTITCKASQDINKYIAWFQQKPGKAPKLVIHYTSILQPGVPSRFSGVGSGTDYTFTISSLQPEDIATYYCLQYDNLPWTFGGGTKVEIK

SEQ ID NO: 80 - DNA, 324 bp, Homo sapiens
  source 1..324: mol_type = other DNA
  CDS 1..324
atggcccgcgctgctctctccgccgcccccagcaatccccggctcctgcgagtggcactgctgctcctgctcctggtagccgctggccggcgcgcagcaggagcgtccgtggccactgaactgcgctgccagtgcttgcagaccctgcagggaattcaccccaagaacatccaaagtgtgaacgtgaagtcccccggaccccactgcgcccaaaccgaagtcatagccacactcaagaatgggcggaaagcttgcctcaatcctgcatcccccatagttaagaaaatcatcgaaaagatgctgaacagtgacaaatccaactag

SEQ ID NO: 81 - protein, 107 aa, Homo sapiens
MARAALSAAPSNPRLLRVALLLLLLVAAGRRAAGASVATELRCQCLQTLQGIHPKNIQSVNVKSPGPHCAQTEVIATLKNGRKACLNPASPIVKKIIEKMLNSDKSN

SEQ ID NO: 82 - protein, 107 aa, Macaca fascicularis
MARAALSAAPSNPRFLQVALLLLLLVATGRRAAGASVVTELRCQCLQTLQGIHPKNIQSVNVKAPGPHCAETEVIATLKNGQKACLNPASPMVQKIIKKMLNCDKSN